European Patent Application EP 4 703 372 A1, published March 4, 2026. Title: IMMUNOGLOBULIN-BINDING PROTEIN. Applicant: TOSOH corporation. Application JP PCT/JP2024/015488, filed April 18, 2024. The sequence listing filed with the application follows.

SEQUENCE LISTING (107 sequences)

SEQ ID NO: 1 - protein, 70 aa, Finegoldia magna
  source 1..70: note = FpL_C3(FpL domain C3)
ETPEEPKEEVTIKVNLIFADGKIQTAEFKGTFEEATAKAYAYANLLAKENGEYTADLEDGGNTINIKFAG

SEQ ID NO: 2 - DNA, 210 bp, Finegoldia magna
  source 1..210: mol_type = genomic DNA
  misc_feature 1..210: note = FpL_C3_DNA
gaaactcccgaagaaccaaaagaagaagttacgattaaggttaacttaatcttcgccgacggtaagattcagacagctgaatttaagggaacattcgaagaagcgaccgcgaaagcatacgcgtacgccaacctgctggcgaaagaaaacggtgagtataccgccgatttagaagatggcggcaatacgatcaatatcaagtttgcgggt

SEQ ID NO: 3 - DNA, 20 bp, synthetic construct
  misc_feature 1..20: note = PCR forward primer
  source 1..20: mol_type = other DNA
  misc_feature 1..20: note = T7 promoter
taatacgactcactataggg

SEQ ID NO: 4 - DNA, 19 bp, synthetic construct
  source 1..19: mol_type = other DNA
  misc_feature 1..19: note = T7 terminator
tatgctagttattgctcag

SEQ ID NO: 5 - protein, 70 aa, synthetic construct
  REGION 1..70: note = FpL_C3 N62Y
ETPEEPKEEVTIKVNLIFADGKIQTAEFKGTFEEATAKAYAYANLLAKENGEYTADLEDGGYTINIKFAG

SEQ ID NO: 6 - protein, 70 aa, synthetic construct
  REGION 1..70: note = FpL_C3_I17F,N50S
ETPEEPKEEVTIKVNLFFADGKIQTAEFKGTFEEATAKAYAYANLLAKESGEYTADLEDGGNTINIKFAG

SEQ ID NO: 7 - protein, 70 aa, synthetic construct
  REGION 1..70: note = FpL_C3_K22R,K29R,N44S
ETPEEPKEEVTIKVNLIFADGRIQTAEFRGTFEEATAKAYAYASLLAKENGEYTADLEDGGNTINIKFAG

SEQ ID NO: 8 - protein, 70 aa, synthetic construct
  REGION 1..70: note = FpL_C3_E8G,E52V,N62Y
ETPEEPKGEVTIKVNLIFADGKIQTAEFKGTFEEATAKAYAYANLLAKENGVYTADLEDGGYTINIKFAG

SEQ ID NO: 9 - protein, 70 aa, synthetic construct
  REGION 1..70: note = FpL_C3_E49V
ETPEEPKEEVTIKVNLIFADGKIQTAEFKGTFEEATAKAYAYANLLAKVNGEYTADLEDGGNTINIKFAG

SEQ ID NO: 10 - protein, 70 aa, synthetic construct
  REGION 1..70: note = FpL_C3_K22R
ETPEEPKEEVTIKVNLIFADGRIQTAEFKGTFEEATAKAYAYANLLAKENGEYTADLEDGGNTINIKFAG

SEQ ID NO: 11 - protein, 70 aa, synthetic construct
  REGION 1..70: note = FpL_C3_N50Y,E52G (FpL_C3 2a)
ETPEEPKEEVTIKVNLIFADGKIQTAEFKGTFEEATAKAYAYANLLAKEYGGYTADLEDGGNTINIKFAG

SEQ ID NO: 12 - protein, 70 aa, synthetic construct
  REGION 1..70: note = FpL_C3_E27G,A41T,N50K,N65Y
ETPEEPKEEVTIKVNLIFADGKIQTAGFKGTFEEATAKAYTYANLLAKEKGEYTADLEDGGNTIYIKFAG

SEQ ID NO: 13 - protein, 70 aa, synthetic construct
  REGION 1..70: note = FpL_C3_N50S
ETPEEPKEEVTIKVNLIFADGKIQTAEFKGTFEEATAKAYAYANLLAKESGEYTADLEDGGNTINIKFAG

SEQ ID NO: 14 - protein, 70 aa, synthetic construct
  REGION 1..70: note = FpL_C3_E5V
ETPEVPKEEVTIKVNLIFADGKIQTAEFKGTFEEATAKAYAYANLLAKENGEYTADLEDGGNTINIKFAG

SEQ ID NO: 15 - protein, 70 aa, synthetic construct
  REGION 1..70: note = FpL_C3_P3S,N50D,T54I
ETSEEPKEEVTIKVNLIFADGKIQTAEFKGTFEEATAKAYAYANLLAKEDGEYIADLEDGGNTINIKFAG

SEQ ID NO: 16 - protein, 70 aa, synthetic construct
  REGION 1..70: note = FpL_C3_E52G
ETPEEPKEEVTIKVNLIFADGKIQTAEFKGTFEEATAKAYAYANLLAKENGGYTADLEDGGNTINIKFAG

SEQ ID NO: 17 - protein, 70 aa, synthetic construct
  REGION 1..70: note = FpL_C3_K38R
ETPEEPKEEVTIKVNLIFADGKIQTAEFKGTFEEATARAYAYANLLAKENGEYTADLEDGGNTINIKFAG

SEQ ID NO: 18 - protein, 70 aa, synthetic construct
  REGION 1..70: note = FpL_C3KR
ETPEEPREEVTIRVNLIFADGRIQTAEFRGTFEEATARAYAYANLLARENGEYTADLEDGGNTINIRFAG

SEQ ID NO: 19 - protein, 70 aa, synthetic construct
  REGION 1..70: note = FpL_C3KR 3a
ETPEEPREEVTIRVNLIFADGRIQTAEFRGTFEEATARAYAYANLLAREYGGYTADLEDGGYTINIRFAG

SEQ ID NO: 20 - protein, 70 aa, synthetic construct
  REGION 1..70: note = FpL_C3KX
ETPEEPAEEVTIRVNLIFADGQIQTAEFIGTFEEATARAYAYANLLARENGEYTADLEDGGNTINIRFAG

SEQ ID NO: 21 - protein, 70 aa, synthetic construct
  REGION 1..70: note = FpL_C3KX 3a
ETPEEPAEEVTIRVNLIFADGQIQTAEFIGTFEEATARAYAYANLLAREYGGYTADLEDGGYTINIRFAG

SEQ ID NO: 22 - protein, 70 aa, synthetic construct
  REGION 1..70: note = FpL_C3KX 3a_E4K
ETPKEPAEEVTIRVNLIFADGQIQTAEFIGTFEEATARAYAYANLLAREYGGYTADLEDGGYTINIRFAG

SEQ ID NO: 23 - protein, 70 aa, synthetic construct
  REGION 1..70: note = FpL_C3KX 3a_K22T
ETPEEPAEEVTIRVNLIFADGTIQTAEFIGTFEEATARAYAYANLLAREYGGYTADLEDGGYTINIRFAG

SEQ ID NO: 24 - protein, 70 aa, synthetic construct
  REGION 1..70: note = FpL_C3KX 3a_E27R
ETPEEPAEEVTIRVNLIFADGQIQTARFIGTFEEATARAYAYANLLAREYGGYTADLEDGGYTINIRFAG

SEQ ID NO: 25 - protein, 70 aa, synthetic construct
  REGION 1..70: note = FpL_C3KX 3a_T36A
ETPEEPAEEVTIRVNLIFADGQIQTAEFIGTFEEAAARAYAYANLLAREYGGYTADLEDGGYTINIRFAG

SEQ ID NO: 26 - protein, 70 aa, synthetic construct
  REGION 1..70: note = FpL_C3KX 3a_E49D(FpL_C3KX 4h)
ETPEEPAEEVTIRVNLIFADGQIQTAEFIGTFEEATARAYAYANLLARDYGGYTADLEDGGYTINIRFAG

SEQ ID NO: 27 - DNA, 210 bp, synthetic construct
  misc_feature 1..210: note = FpL_C3KX 4h DNA
  source 1..210: mol_type = other DNA
gaaacaccagaagagccagcggaagaagttaccattcgcgtgaatctgatctttgccgacggtcagattcagaccgctgaattcattggtacattcgaagaagccacagctcgtgcctatgcttatgcgaatttgctggcccgtgattatggtggctatacggcggacctggaagatggcgggtataccatcaacatccgctttgcggga

SEQ ID NO: 28 - protein, 70 aa, synthetic construct
  REGION 1..70: note = FpL_C3KX 4h_E9V
ETPEEPAEVVTIRVNLIFADGQIQTAEFIGTFEEATARAYAYANLLARDYGGYTADLEDGGYTINIRFAG

SEQ ID NO: 29 - protein, 70 aa, synthetic construct
  REGION 1..70: note = FpL_C3KX 4h_K22R(FpL_C3KX 4i)
ETPEEPAEEVTIRVNLIFADGRIQTAEFIGTFEEATARAYAYANLLARDYGGYTADLEDGGYTINIRFAG

SEQ ID NO: 30 - protein, 70 aa, synthetic construct
  REGION 1..70: note = FpL_C3KX 4h_Y53F
ETPEEPAEEVTIRVNLIFADGQIQTAEFIGTFEEATARAYAYANLLARDYGGFTADLEDGGYTINIRFAG

SEQ ID NO: 31 - protein, 70 aa, synthetic construct
  REGION 1..70: note = FpL_C3KX 4h_T54M
ETPEEPAEEVTIRVNLIFADGQIQTAEFIGTFEEATARAYAYANLLARDYGGYMADLEDGGYTINIRFAG

SEQ ID NO: 32 - protein, 70 aa, synthetic construct
  REGION 1..70: note = FpL_C3KX 4h_A69T
ETPEEPAEEVTIRVNLIFADGQIQTAEFIGTFEEATARAYAYANLLARDYGGYTADLEDGGYTINIRFTG

SEQ ID NO: 33 - protein, 70 aa, synthetic construct
  REGION 1..70: note = FpL_C3KX 4i_Y53F(FpL_C3KX 5e)
ETPEEPAEEVTIRVNLIFADGRIQTAEFIGTFEEATARAYAYANLLARDYGGFTADLEDGGYTINIRFAG

SEQ ID NO: 34 - DNA, 210 bp, synthetic construct
  misc_feature 1..210: note = FpL_C3KX 5e DNA
  source 1..210: mol_type = other DNA
gaaacaccagaagagccagcggaagaagttaccattcgcgtgaatctgatctttgccgacggtcggattcagaccgctgaattcattggtacattcgaagaagccacagctcgtgcctatgcttatgcgaatttgctggcccgtgattatggtggctttacggcggacctggaagatggcgggtataccatcaacatccgctttgcggga

SEQ ID NO: 35 - protein, 70 aa, synthetic construct
  REGION 1..70: note = FpL_C3KX 5e_E1V
VTPEEPAEEVTIRVNLIFADGRIQTAEFIGTFEEATARAYAYANLLARDYGGFTADLEDGGYTINIRFAG

SEQ ID NO: 36 - protein, 70 aa, synthetic construct
  REGION 1..70: note = FpL_C3KX 5e_E4G
ETPGEPAEEVTIRVNLIFADGRIQTAEFIGTFEEATARAYAYANLLARDYGGFTADLEDGGYTINIRFAG

SEQ ID NO: 37 - protein, 70 aa, synthetic construct
  REGION 1..70: note = FpL_C3KX 5e_K7S
ETPEEPSEEVTIRVNLIFADGRIQTAEFIGTFEEATARAYAYANLLARDYGGFTADLEDGGYTINIRFAG

SEQ ID NO: 38 - protein, 70 aa, synthetic construct
  REGION 1..70: note = FpL_C3KX 5e_G21R
ETPEEPAEEVTIRVNLIFADRRIQTAEFIGTFEEATARAYAYANLLARDYGGFTADLEDGGYTINIRFAG

SEQ ID NO: 39 - protein, 70 aa, synthetic construct
  REGION 1..70: note = FpL_C3KX 5e_E52D
ETPEEPAEEVTIRVNLIFADGRIQTAEFIGTFEEATARAYAYANLLARDYGDFTADLEDGGYTINIRFAG

SEQ ID NO: 40 - protein, 70 aa, synthetic construct
  REGION 1..70: note = FpL_C3KX 5e_P6S
ETPEESAEEVTIRVNLIFADGRIQTAEFIGTFEEATARAYAYANLLARDYGGFTADLEDGGYTINIRFAG

SEQ ID NO: 41 - protein, 70 aa, synthetic construct
  REGION 1..70: note = FpL_C3KR_K38E
ETPEEPREEVTIRVNLIFADGRIQTAEFRGTFEEATAEAYAYANLLARENGEYTADLEDGGNTINIRFAG

SEQ ID NO: 42 - protein, 70 aa, synthetic construct
  REGION 1..70: note = FpL_C3KX 5e_E4G,K38E,E52D(FpL_C3KX 7d)
ETPGESAEEVTIRVNLIFADGRIQTAEFIGTFEEATAEAYAYANLLARDYGDFTADLEDGGYTINIRFAG

SEQ ID NO: 43 - DNA, 210 bp, synthetic construct
  misc_feature 1..210: note = FpL_C3KX 7d DNA
  source 1..210: mol_type = other DNA
gaaacaccaggagagtcagcggaagaagttaccattcgcgtgaatctgatctttgccgacggtcggattcagaccgctgaattcattggtacattcgaagaagccacagctgaagcctatgcttatgcgaatttgctggcccgtgattatggtgactttacggcggacctggaagatggcgggtataccatcaacatccgctttgcggga

SEQ ID NO: 44 - protein, 70 aa, synthetic construct
  REGION 1..70: note = FpL_C3KX 7d_A69V
ETPGESAEEVTIRVNLIFADGRIQTAEFIGTFEEATAEAYAYANLLARDYGDFTADLEDGGYTINIRFVG

SEQ ID NO: 45 - protein, 70 aa, synthetic construct
  REGION 1..70: note = FpL_C3KX 7d_I29F
ETPGESAEEVTIRVNLIFADGRIQTAEFFGTFEEATAEAYAYANLLARDYGDFTADLEDGGYTINIRFAG

SEQ ID NO: 46 - protein, 70 aa, synthetic construct
  REGION 1..70: note = FpL_C3KX 7d_E8G,E33V
ETPGESAGEVTIRVNLIFADGRIQTAEFIGTFVEATAEAYAYANLLARDYGDFTADLEDGGYTINIRFAG

SEQ ID NO: 47 - DNA, 27 bp, synthetic construct
  misc_feature 1..27: note = I23X forward primer 1
  misc_feature 7: note = n is a, c, g, or t
  source 1..27: mol_type = other DNA
ggtcggndtcagaccgctgaattcatt

SEQ ID NO: 48 - DNA, 27 bp, synthetic construct
  misc_feature 1..27: note = I23X forward primer 2
  source 1..27: mol_type = other DNA
ggtcggvhgcagaccgctgaattcatt

SEQ ID NO: 49 - DNA, 27 bp, synthetic construct
  misc_feature 1..27: note = I23X forward primer 3
  source 1..27: mol_type = other DNA
ggtcggtggcagaccgctgaattcatt

SEQ ID NO: 50 - DNA, 27 bp, synthetic construct
  misc_feature 1..27: note = I23X reverse primer 1
  misc_feature 9: note = n is a, c, g, or t
  source 1..27: mol_type = other DNA
accgtcahnccgaccgtcggcaaagat

SEQ ID NO: 51 - DNA, 27 bp, synthetic construct
  misc_feature 1..27: note = I23X reverse primer 2
  source 1..27: mol_type = other DNA
accgtccdbccgaccgtcggcaaagat

SEQ ID NO: 52 - DNA, 27 bp, synthetic construct
  misc_feature 1..27: note = A41X forward primer 1
  source 1..27: mol_type = other DNA
accgtcccaccgaccgtcggcaaagat

SEQ ID NO: 53 - protein, 70 aa, synthetic construct
  REGION 1..70: note = FpL_C3KX 7d_I23R
ETPGESAEEVTIRVNLIFADGRRQTAEFIGTFEEATAEAYAYANLLARDYGDFTADLEDGGYTINIRFAG

SEQ ID NO: 54 - DNA, 27 bp, synthetic construct
  misc_feature 1..27: note = A41X forward primer 1
  misc_feature 7: note = n is a, c, g, or t
  source 1..27: mol_type = other DNA
gcctatndttatgcgaatttgctggcc

SEQ ID NO: 55 - DNA, 27 bp, synthetic construct
  misc_feature 1..27: note = A41X forward primer 2
  source 1..27: mol_type = other DNA
gcctatvhgtatgcgaatttgctggcc

SEQ ID NO: 56 - DNA, 27 bp, synthetic construct
  misc_feature 1..27: note = A41X forward primer 3
  source 1..27: mol_type = other DNA
gcctattggtatgcgaatttgctggcc

SEQ ID NO: 57 - DNA, 27 bp, synthetic construct
  misc_feature 1..27: note = A41X reverse primer 1
  misc_feature 9: note = n is a, c, g, or t
  source 1..27: mol_type = other DNA
ggcttcahnataggcttcagctgtggc

SEQ ID NO: 58 - DNA, 27 bp, synthetic construct
  misc_feature 1..27: note = A41X reverse primer 2
  source 1..27: mol_type = other DNA
ggcttccdbataggcttcagctgtggc

SEQ ID NO: 59 - DNA, 27 bp, synthetic construct
  misc_feature 1..27: note = A41X reverse primer 3
  source 1..27: mol_type = other DNA
ggcttcccaataggcttcagctgtggc

SEQ ID NO: 60 - protein, 70 aa, synthetic construct
  REGION 1..70: note = FpL_C3KX 7d_A41I
ETPGESAEEVTIRVNLIFADGRIQTAEFIGTFEEATAEAYIYANLLARDYGDFTADLEDGGYTINIRFAG

SEQ ID NO: 61 - protein, 70 aa, synthetic construct
  REGION 1..70: note = FpL_C3KX 7d_A41Y
ETPGESAEEVTIRVNLIFADGRIQTAEFIGTFEEATAEAYYYANLLARDYGDFTADLEDGGYTINIRFAG

SEQ ID NO: 62 - DNA, 27 bp, synthetic construct
  misc_feature 1..27: note = E52X forward primer 1
  misc_feature 7: note = n is a, c, g, or t
  source 1..27: mol_type = other DNA
tatggtndttttacggcggacctggaa

SEQ ID NO: 63 - DNA, 27 bp, synthetic construct
  misc_feature 1..27: note = E52X forward primer 2
  source 1..27: mol_type = other DNA
tatggtvhgtttacggcggacctggaa

SEQ ID NO: 64 - DNA, 27 bp, synthetic construct
  misc_feature 1..27: note = E52X forward primer 3
  source 1..27: mol_type = other DNA
tatggttggtttacggcggacctggaa

SEQ ID NO: 65 - DNA, 27 bp, synthetic construct
  misc_feature 1..27: note = E52X reverse primer 1
  misc_feature 9: note = n is a, c, g, or t
  source 1..27: mol_type = other DNA
ataatcahnaccataatcacgggccag

SEQ ID NO: 66 - DNA, 27 bp, synthetic construct
  misc_feature 1..27: note = E52X reverse primer 2
  source 1..27: mol_type = other DNA
ataatccdbaccataatcacgggccag

SEQ ID NO: 67 - DNA, 27 bp, synthetic construct
  misc_feature 1..27: note = E52X reverse primer 3
  source 1..27: mol_type = other DNA
ataatcccaaccataatcacgggccag

SEQ ID NO: 68 - protein, 70 aa, synthetic construct
  REGION 1..70: note = FpL_C3KX 7d_E52L
ETPGESAEEVTIRVNLIFADGRIQTAEFIGTFEEATAEAYAYANLLARDYGLFTADLEDGGYTINIRFAG

SEQ ID NO: 69 - protein, 70 aa, synthetic construct
  REGION 1..70: note = FpL_C3KX 7d_E52V
ETPGESAEEVTIRVNLIFADGRIQTAEFIGTFEEATAEAYAYANLLARDYGVFTADLEDGGYTINIRFAG

SEQ ID NO: 70 - protein, 70 aa, synthetic construct
  REGION 1..70: note = FpL_C3KX 7d_E52L,A69V(FpL_C3KX 8b)
ETPGESAEEVTIRVNLIFADGRIQTAEFIGTFEEATAEAYAYANLLARDYGLFTADLEDGGYTINIRFVG

SEQ ID NO: 71 - DNA, 27 bp, synthetic construct
  source 1..27: mol_type = other DNA
  misc_feature 1..27: note = K22X forward primer 1
gacggtndtattcagaccgccgaattc

SEQ ID NO: 72 - DNA, 27 bp, synthetic construct
  source 1..27: mol_type = other DNA
  misc_feature 1..27: note = K22X forward primer 2
gacggtvhgattcagaccgccgaattc

SEQ ID NO: 73 - DNA, 27 bp, synthetic construct
  source 1..27: mol_type = other DNA
  misc_feature 1..27: note = K22X forward primer 3
acagcttgggcctatgcttatgcgaat

SEQ ID NO: 74 - DNA, 27 bp, synthetic construct
  source 1..27: mol_type = other DNA
  misc_feature 1..27: note = K22X reverse primer 1
ctgaatahnaccgtcggcaaagatcag

SEQ ID NO: 75 - DNA, 27 bp, synthetic construct
  source 1..27: mol_type = other DNA
  misc_feature 1..27: note = K22X reverse primer 2
ctgaatcdbaccgtcggcaaagatcag

SEQ ID NO: 76 - DNA, 27 bp, synthetic construct
  source 1..27: mol_type = other DNA
  misc_feature 1..27: note = K22X reverse primer 3
ctgaatccaaccgtcggcaaagatcag

SEQ ID NO: 77 - DNA, 27 bp, synthetic construct
  source 1..27: mol_type = other DNA
  misc_feature 1..27: note = K38X forward primer 1
acagctndtgcctatgcttatgcgaat

SEQ ID NO: 78 - DNA, 27 bp, synthetic construct
  source 1..27: mol_type = other DNA
  misc_feature 1..27: note = K38X forward primer 2
acagctvhggcctatgcttatgcgaat

SEQ ID NO: 79 - DNA, 27 bp, synthetic construct
  source 1..27: mol_type = other DNA
  misc_feature 1..27: note = K38X forward primer 3
acagcttgggcctatgcttatgcgaat

SEQ ID NO: 80 - DNA, 27 bp, synthetic construct
  source 1..27: mol_type = other DNA
  misc_feature 1..27: note = K38X reverse primer 1
ataggcahnagctgtggcttcttcgaa

SEQ ID NO: 81 - DNA, 27 bp, synthetic construct
  source 1..27: mol_type = other DNA
  misc_feature 1..27: note = K38X reverse primer 2
ataggccdbagctgtggcttcttcgaa

SEQ ID NO: 82 - DNA, 27 bp, synthetic construct
  source 1..27: mol_type = other DNA
  misc_feature 1..27: note = K38X reverse primer 3
ataggcccaagctgtggcttcttcgaa

SEQ ID NO: 83 - DNA, 27 bp, synthetic construct
  source 1..27: mol_type = other DNA
  misc_feature 1..27: note = Y42X forward primer 1
tatgctndtgcgaatttgctggcccgt

SEQ ID NO: 84 - DNA, 27 bp, synthetic construct
  source 1..27: mol_type = other DNA
  misc_feature 1..27: note = Y42X forward primer 2
tatgctvhggcgaatttgctggcccgt

SEQ ID NO: 85 - DNA, 27 bp, synthetic construct
  source 1..27: mol_type = other DNA
  misc_feature 1..27: note = Y42X forward primer 3
tatgcttgggcgaatttgctggcccgt

SEQ ID NO: 86 - DNA, 27 bp, synthetic construct
  source 1..27: mol_type = other DNA
  misc_feature 1..27: note = Y42X reverse primer 1
attcgcahnagcataggcttcagctgt

SEQ ID NO: 87 - DNA, 27 bp, synthetic construct
  source 1..27: mol_type = other DNA
  misc_feature 1..27: note = Y42X reverse primer 2
attcgccdbagcataggcttcagctgt

SEQ ID NO: 88 - DNA, 27 bp, synthetic construct
  source 1..27: mol_type = other DNA
  misc_feature 1..27: note = Y42X reverse primer 3
attcgcccaagcataggcttcagctgt

SEQ ID NO: 89 - DNA, 27 bp, synthetic construct
  source 1..27: mol_type = other DNA
  misc_feature 1..27: note = N44X forward primer 1
tatgcgndtttgctggcccgtgattat

SEQ ID NO: 90 - DNA, 27 bp, synthetic construct
  source 1..27: mol_type = other DNA
  misc_feature 1..27: note = N44X forward primer 2
tatgcgvhgttgctggcccgtgattat

SEQ ID NO: 91 - DNA, 27 bp, synthetic construct
  source 1..27: mol_type = other DNA
  misc_feature 1..27: note = N44X forward primer 3
tatgcgtggttgctggcccgtgattat

SEQ ID NO: 92 - DNA, 27 bp, synthetic construct
  source 1..27: mol_type = other DNA
  misc_feature 1..27: note = N44X reverse primer 1
cagcaaahncgcataagcataggcttc

SEQ ID NO: 93 - DNA, 27 bp, synthetic construct
  source 1..27: mol_type = other DNA
  misc_feature 1..27: note = N44X reverse primer 2
cagcaacdbcgcataagcataggcttc

SEQ ID NO: 94 - DNA, 27 bp, synthetic construct
  source 1..27: mol_type = other DNA
  misc_feature 1..27: note = N44X reverse primer 3
cagcaaccacgcataagcataggcttc

SEQ ID NO: 95 - protein, 70 aa, synthetic construct
  REGION 1..70: note = FpL_C3KX 8b_K22E
ETPGESAEEVTIRVNLIFADGEIQTAEFIGTFEEATAEAYAYANLLARDYGLFTADLEDGGYTINIRFVG

SEQ ID NO: 96 - protein, 70 aa, synthetic construct
  REGION 1..70: note = FpL_C3KX 8b_K38P
ETPGESAEEVTIRVNLIFADGRIQTAEFIGTFEEATAPAYAYANLLARDYGLFTADLEDGGYTINIRFVG

SEQ ID NO: 97 - protein, 70 aa, synthetic construct
  REGION 1..70: note = FpL_C3KX 8b_K38D
ETPGESAEEVTIRVNLIFADGRIQTAEFIGTFEEATADAYAYANLLARDYGLFTADLEDGGYTINIRFVG

SEQ ID NO: 98 - protein, 70 aa, synthetic construct
  REGION 1..70: note = FpL_C3KX 8b_Y42W
ETPGESAEEVTIRVNLIFADGRIQTAEFIGTFEEATAEAYAWANLLARDYGLFTADLEDGGYTINIRFVG

SEQ ID NO: 99 - protein, 70 aa, synthetic construct
  REGION 1..70: note = FpL_C3KX 8b_Y42F
ETPGESAEEVTIRVNLIFADGRIQTAEFIGTFEEATAEAYAFANLLARDYGLFTADLEDGGYTINIRFVG

SEQ ID NO: 100 - protein, 70 aa, synthetic construct
  REGION 1..70: note = FpL_C3KX 8b_Y42H
ETPGESAEEVTIRVNLIFADGRIQTAEFIGTFEEATAEAYAHANLLARDYGLFTADLEDGGYTINIRFVG

SEQ ID NO: 101 - protein, 70 aa, synthetic construct
  REGION 1..70: note = FpL_C3KX 8b_N44P
ETPGESAEEVTIRVNLIFADGRIQTAEFIGTFEEATAEAYAYAPLLARDYGLFTADLEDGGYTINIRFVG

SEQ ID NO: 102 - protein, 70 aa, synthetic construct
  REGION 1..70: note = FpL_C3KX 8b_K38D,Y42H
ETPGESAEEVTIRVNLIFADGRIQTAEFIGTFEEATADAYAHANLLARDYGLFTADLEDGGYTINIRFVG

SEQ ID NO: 103 - DNA, 210 bp, synthetic construct
  source 1..210: mol_type = other DNA
  misc_feature 1..210: note = FpL_C3KX 8b_Y42H DNA
gaaacaccaggagagtcagcggaagaagttaccattcgcgtgaatctgatctttgccgacggtcggattcagaccgccgaattcattggtacattcgaagaagccacagctgaagcctatgctcatgcgaatttgctggcccgtgattatggtctgtttacggcggacctggaagatggcgggtataccatcaacatccgctttgtggga

SEQ ID NO: 104 - DNA, 27 bp, synthetic construct
  source 1..27: mol_type = other DNA
  misc_feature 1..27: note = PCR forward primer
acagctgatgcctatgctcatgcgaat

SEQ ID NO: 105 - DNA, 27 bp, synthetic construct
  source 1..27: mol_type = other DNA
  misc_feature 1..27: note = PCR reverse primer
ataggcatcagctgtggcttcttcgaa

SEQ ID NO: 106 - protein, 960 aa, Finegoldia magna
  REGION 1..960: note = GenBank No. AAA67503
MKINKKLLMAALAGAIVVGGGANAYAAEEDNTDNNLSMDEISDAYFDYHGDVSDSVDPVEEEIDEALAKALAEAKETAKKHIDSLNHLSETAKKLAKNDIDSATTINAINDIVARADVMERKTAEKEEAEKLAAAKETAKKHIDELKHLADKTKELAKRDIDSATTINAINDIVARADVMERKTAEKEEAEKLAAAKETAKKHIDELKHLADKTKELAKRDIDSATTIDAINDIVARADVMERKLSEKETPEPEEEVTIKANLIFADGSTQNAEFKGTFAKAVSDAYAYADALKKDNGEYTVDVADKGLTLNIKFAGKKEKPEEPKEEVTIKVNLIFADGKTQTAEFKGTFEEATAKAYAYADLLAKENGEYTADLEDGGNTINIKFAGKETPETPEEPKEEVTIKVNLIFADGKIQTAEFKGTFEEATAKAYAYANLLAKENGEYTADLEDGGNTINIKFAGKETPETPEEPKEEVTIKVNLIFADGKTQTAEFKGTFEEATAEAYRYADLLAKVNGEYTADLEDGGYTINIKFAGKEQPGENPGITIDEWLLKNAKEEAIKELKEAGITSDLYFSLINKAKTVEGVEALKNEILKAHAGEETPELKDGYATYEEAEAAAKEALKNDDVNNAYEIVQGADGRYYYVLKIEVADEEEPGEDTPEVQEGYATYEEAEAAAKEALKEDKVNNAYEVVQGADGRYYYVLKIEDKEDEQPGEEPGENPGITIDEWLLKNAKEDAIKELKEAGISSDIYFDAINKAKTVEGVEALKNEILKAHAEKPGENPGITIDEWLLKNAKEAAIKELKEAGITAEYLFNLINKAKTVEGVESLKNEILKAHAEKPGENPGITIDEWLLKNAKEDAIKELKEAGITSDIYFDAINKAKTIEGVEALKNEILKAHKKDEEPGKKPGEDKKPEDKKPGEDKKPEDKKPGEDKKPEDKKPGKTDKDSPNKKKKAK

SEQ ID NO: 107 - DNA, 18 bp, synthetic construct
  source 1..18: mol_type = other DNA
  misc_feature 1..18: note = 6His DNA
catcaccaccatcaccac